European Patent Specification EP 3 689 898 B1, published April 29, 2026. Title: Long-acting conjugates of GLP-2 derivatives. Applicant: HANMI PHARM. CO., LTD. The sequence listing filed with the application follows.

SEQUENCE LISTING (9 sequences)

SEQ ID NO: 1 - protein, 33 aa, Homo sapiens
HADGSFSDEMNTILDNLAARDFINWLIQTKITD

SEQ ID NO: 2 - protein, 34 aa, Artificial Sequence
  GLP-2 derivative
  MISC_FEATURE (1): Xaa is imidazoacetyldeshistidine
XGDGSFSDEMNTILDNLAARDFINWLIQTKITDC

SEQ ID NO: 3 - protein, 34 aa, Artificial Sequence
  GLP-2 derivative
  MISC_FEATURE (1): Xaa is imidazoacetyldeshistidine
XGDGSFSDEMNTILDNLAARDFINWLIQTKITDK

SEQ ID NO: 4 - protein, 34 aa, Artificial Sequence
  GLP-2 derivative
  MISC_FEATURE (1): Xaa is imidazoacetyldeshistidine
XGDGSFSDEMNTILDNLAARDFINWLIQTRITDK

SEQ ID NO: 5 - protein, 34 aa, Artificial Sequence
  GLP-2 derivative
  MISC_FEATURE (1): Xaa is imidazoacetyldeshistidine
  MISC_FEATURE (34): Xaa is 6-azidolysine
XGDGSFSDEMNTILDNLAARDFINWLIQTKITDX

SEQ ID NO: 6 - protein, 34 aa, Artificial Sequence
  GLP-2 derivative
  MISC_FEATURE (1): Xaa is imidazoacetyldeshistidine
XGDGSFSDEMNTILDNLAARDFINWLIQTRITDC

SEQ ID NO: 7 - protein, 34 aa, Artificial Sequence
  GLP-2 derivative
  MISC_FEATURE (1): Xaa is imidazoacetyldeshistidine
  MISC_FEATURE (2): Xaa is Aib(2-aminoisobutyric acid)
XXDGSFSDEMNTILDNLAARDFINWLIQTKITDC

SEQ ID NO: 8 - protein, 34 aa, Artificial Sequence
  GLP-2 derivative
  MISC_FEATURE (2): Xaa is Aib(2-aminoisobutyric acid)
HXDGSFSDEMNTILDNLAARDFINWLIQTKITDC

SEQ ID NO: 9 - protein, 34 aa, Artificial Sequence
  GLP-2 derivative
  MISC_FEATURE (1): Xaa = Histidine, imidazoacetyldeshistidine, desaminohistidine, beta-hydroxyimidazopropionyldeshistidine, N-dimethylhistidine, or beta-carboxyimidazopropionyldeshistidine
  MISC_FEATURE (2): Xaa is Alanine, Glycine, or Aib(2-aminoisobutyric acid)
  MISC_FEATURE (30): Xaa is Lysine, or Arginine
  MISC_FEATURE (34): Xaa is absent, Lysine, Arginine, Glutamine, Histidine, 6-azidolysine, or Cysteine
XXDGSFSDEMNTILDNLAARDFINWLIQTXITDX